European Patent Application EP 4 570 812 A1, published June 18, 2025. Title: エステル化タンパク質及びその製造方法. Applicant: Ｓｐｉｂｅｒ株式会社. The sequence listing filed with the application follows.

SEQUENCE LISTING (12 sequences)

SEQ ID NO: 1 - protein, 2375 aa, synthetic construct
  source 1..2375: note = PRT799
MHHHHHHSSGSSGPGQQGPYGPGASAAAAAGQNGPGSGQQGPGQSGQYGPGQQGPGQQGPGSSAAAAAGPGQYGPGQQGPSASAAAAAGPGSGQQGPGASGQYGPGQQGPGQQGPGSSAAAAAGQYGSGPGQQGPYGSAAAAAGPGSGQYGQGPYGPGASGPGQYGPGQQGPSASAAAAAGSGQQGPGQYGPYASAAAAAGQYGSGPGQQGPYGPGQSGSGQQGPGQQGPYASAAAAAGPGQQGPYGPGSSAAAAAGQYGYGPGQQGPYGPGASGQNGPGSGQYGPGQQGPGQSAAAAAGPGQQGPYGPGASAAAAAGQYGPGQQGPGQYGPGSSGPGQQGPYGPGSSAAAAAGQYGPGQQGPYGPGQSAAAAAGQYQQGPGQQGPYGPGASGPGQQGPYGPGASAAAAAGPGQYGPGQQGPSASAAAAAGQYGSGPGQYGPYGPGQSGPGSGQQGQGPYGPGASAAAAAGQYGPGQQGPYGPGQSAAAAAGPGSGQYGPGASGQNGPGSGQYGPGQQGPGQSAAAAAGQYQQGPGQQGPYGPGASAAAAAGQYGSGPGQQGPYGPGQSGSGQQGPGQQGPYASAAAAAGPGSGQQGPGASGQQGPYGPGASAAAAAGQNGPGSGQQGPGQSGQYGPGQQGPGQQGPGSSAAAAAGPGQYGPGQQGPSASAAAAAGPGSGQQGPGASGQYGPGQQGPGQQGPGSSAAAAAGQYGSGPGQQGPYGSAAAAAGPGSGQYGQGPYGPGASGPGQYGPGQQGPSASAAAAAGSGQQGPGQYGPYASAAAAAGQYGSGPGQQGPYGPGQSGSGQQGPGQQGPYASAAAAAGPGQQGPYGPGSSAAAAAGQYGYGPGQQGPYGPGASGQNGPGSGQYGPGQQGPGQSAAAAAGPGQQGPYGPGASAAAAAGQYGPGQQGPGQYGPGSSGPGQQGPYGPGSSAAAAAGQYGPGQQGPYGPGQSAAAAAGQYQQGPGQQGPYGPGASGPGQQGPYGPGASAAAAAGPGQYGPGQQGPSASAAAAAGQYGSGPGQYGPYGPGQSGPGSGQQGQGPYGPGASAAAAAGQYGPGQQGPYGPGQSAAAAAGPGSGQYGPGASGQNGPGSGQYGPGQQGPGQSAAAAAGQYQQGPGQQGPYGPGASAAAAAGQYGSGPGQQGPYGPGQSGSGQQGPGQQGPYASAAAAAGPGSGQQGPGASGQQGPYGPGASAAAAAGQNGPGSGQQGPGQSGQYGPGQQGPGQQGPGSSAAAAAGPGQYGPGQQGPSASAAAAAGPGSGQQGPGASGQYGPGQQGPGQQGPGSSAAAAAGQYGSGPGQQGPYGSAAAAAGPGSGQYGQGPYGPGASGPGQYGPGQQGPSASAAAAAGSGQQGPGQYGPYASAAAAAGQYGSGPGQQGPYGPGQSGSGQQGPGQQGPYASAAAAAGPGQQGPYGPGSSAAAAAGQYGYGPGQQGPYGPGASGQNGPGSGQYGPGQQGPGQSAAAAAGPGQQGPYGPGASAAAAAGQYGPGQQGPGQYGPGSSGPGQQGPYGPGSSAAAAAGQYGPGQQGPYGPGQSAAAAAGQYQQGPGQQGPYGPGASGPGQQGPYGPGASAAAAAGPGQYGPGQQGPSASAAAAAGQYGSGPGQYGPYGPGQSGPGSGQQGQGPYGPGASAAAAAGQYGPGQQGPYGPGQSAAAAAGPGSGQYGPGASGQNGPGSGQYGPGQQGPGQSAAAAAGQYQQGPGQQGPYGPGASAAAAAGQYGSGPGQQGPYGPGQSGSGQQGPGQQGPYASAAAAAGPGSGQQGPGASGQQGPYGPGASAAAAAGQNGPGSGQQGPGQSGQYGPGQQGPGQQGPGSSAAAAAGPGQYGPGQQGPSASAAAAAGPGSGQQGPGASGQYGPGQQGPGQQGPGSSAAAAAGQYGSGPGQQGPYGSAAAAAGPGSGQYGQGPYGPGASGPGQYGPGQQGPSASAAAAAGSGQQGPGQYGPYASAAAAAGQYGSGPGQQGPYGPGQSGSGQQGPGQQGPYASAAAAAGPGQQGPYGPGSSAAAAAGQYGYGPGQQGPYGPGASGQNGPGSGQYGPGQQGPGQSAAAAAGPGQQGPYGPGASAAAAAGQYGPGQQGPGQYGPGSSGPGQQGPYGPGSSAAAAAGQYGPGQQGPYGPGQSAAAAAGQYQQGPGQQGPYGPGASGPGQQGPYGPGASAAAAAGPGQYGPGQQGPSASAAAAAGQYGSGPGQYGPYGPGQSGPGSGQQGQGPYGPGASAAAAAGQYGPGQQGPYGPGQSAAAAAGPGSGQYGPGASGQNGPGSGQYGPGQQGPGQSAAAAAGQYQQGPGQQGPYGPGASAAAAAGQYGSGPGQQGPYGPGQSGSGQQGPGQQGPYASAAAAAGPGSGQQGSSVDKLAAALEHHHHHH

SEQ ID NO: 2 - protein, 1190 aa, synthetic construct
  source 1..1190: note = PRT966
MHHHHHHSSGSSGPGVFGPYGPGASAAAAAGINGPGSGVFGPGISGIYGPGVFGPGVFGPGSSAAAAAGPGIYGPGVFGPSASAAAAAGPGSGVFGPGASGIYGPGVFGPGVFGPGSSAAAAAGIYGSGPGVFGPYGSAAAAAGPGSGIYGIGPYGPGASGPGIYGPGVFGPSASAAAAAGSGVFGPGIYGPYASAAAAAGIYGSGPGVFGPYGPGISGSGVFGPGVFGPYASAAAAAGPGVFGPYGPGSSAAAAAGIYGYGPGVFGPYGPGASGINGPGSGIYGPGVFGPGISAAAAAGPGVFGPYGPGASAAAAAGIYGPGVFGPGIYGPGSSGPGVFGPYGPGSSAAAAAGIYGPGVFGPYGPGISAAAAAGIYVFGPGVFGPYGPGASGPGVFGPYGPGASAAAAAGPGIYGPGVFGPSASAAAAAGIYGSGPGIYGPYGPGISGPGSGVFGIGPYGPGASAAAAAGIYGPGVFGPYGPGISAAAAAGPGSGIYGPGASGINGPGSGIYGPGVFGPGISAAAAAGIYVFGPGVFGPYGPGASAAAAAGIYGSGPGVFGPYGPGISGSGVFGPGVFGPYASAAAAAGPGSGVFGPGASGPGVFGPYGPGASAAAAAGINGPGSGVFGPGISGIYGPGVFGPGVFGPGSSAAAAAGPGIYGPGVFGPSASAAAAAGPGSGVFGPGASGIYGPGVFGPGVFGPGSSAAAAAGIYGSGPGVFGPYGSAAAAAGPGSGIYGIGPYGPGASGPGIYGPGVFGPSASAAAAAGSGVFGPGIYGPYASAAAAAGIYGSGPGVFGPYGPGISGSGVFGPGVFGPYASAAAAAGPGVFGPYGPGSSAAAAAGIYGYGPGVFGPYGPGASGINGPGSGIYGPGVFGPGISAAAAAGPGVFGPYGPGASAAAAAGIYGPGVFGPGIYGPGSSGPGVFGPYGPGSSAAAAAGIYGPGVFGPYGPGISAAAAAGIYVFGPGVFGPYGPGASGPGVFGPYGPGASAAAAAGPGIYGPGVFGPSASAAAAAGIYGSGPGIYGPYGPGISGPGSGVFGIGPYGPGASAAAAAGIYGPGVFGPYGPGISAAAAAGPGSGIYGPGASGINGPGSGIYGPGVFGPGISAAAAAGIYVFGPGVFGPYGPGASAAAAAGIYGSGPGVFGPYGPGISGSGVFGPGVFGPYASAAAAAGPGSGVFGPGAS

SEQ ID NO: 3 - protein, 601 aa, synthetic construct
  source 1..601: note = PRT918
MHHHHHHSSGSSGPGVFGPYGPGASAAAAAGINGPGSGVFGPGISGIYGPGVFGPGVFGPGSSAAAAAGPGIYGPGVFGPSASAAAAAGPGSGVFGPGASGIYGPGVFGPGVFGPGSSAAAAAGIYGSGPGVFGPYGSAAAAAGPGSGIYGIGPYGPGASGPGIYGPGVFGPSASAAAAAGSGVFGPGIYGPYASAAAAAGIYGSGPGVFGPYGPGISGSGVFGPGVFGPYASAAAAAGPGVFGPYGPGSSAAAAAGIYGYGPGVFGPYGPGASGINGPGSGIYGPGVFGPGISAAAAAGPGVFGPYGPGASAAAAAGIYGPGVFGPGIYGPGSSGPGVFGPYGPGSSAAAAAGIYGPGVFGPYGPGISAAAAAGIYVFGPGVFGPYGPGASGPGVFGPYGPGASAAAAAGPGIYGPGVFGPSASAAAAAGIYGSGPGIYGPYGPGISGPGSGVFGIGPYGPGASAAAAAGIYGPGVFGPYGPGISAAAAAGPGSGIYGPGASGINGPGSGIYGPGVFGPGISAAAAAGIYVFGPGVFGPYGPGASAAAAAGIYGSGPGVFGPYGPGISGSGVFGPGVFGPYASAAAAAGPGSGVFGPGAS

SEQ ID NO: 4 - protein, 608 aa, synthetic construct
  source 1..608: note = PRT313
MHHHHHHSSGSSGPGGQGPYGPGASAAAAAGGNGPGSGQQGPGGSAAAAAGGYGPGGQGPGQQGPGSSAAAAAGPGGYGPGGQGPSASAAAAAGPGSGQQGPGASAAAAAGGYGPGGQGPGQQGPGSSAAAAAGGYGSGPGQQGPYGSAAAAAGPGSGGYGQGPYGPGASAAAAAGPGGYGPGGQGPSASAAAAAGSGQQGPGGYGPYASAAAAAGGYGSGPGQQGPYGPGGSAAAAAGSGQQGPGQQGPYASAAAAAGPGGQGPYGPGSSAAAAAGGYGYGPGGQGPYGPGASAAAAAGGNGPGSGGYGPGQQGPGGSAAAAAGPGGQGPYGPGASAAAAAGGYGPGGQGPGGYGPGSSAAAAAGPGGQGPYGPGSSAAAAAGGYGPGQQGPYGPGGSAAAAAGGYQQGPGGQGPYGPGASAAAAAGPGGQGPYGPGASAAAAAGPGGYGPGGQGPSASAAAAAGGYGSGPGGYGPYGPGGSAAAAAGPGSGQQGQGPYGPGASAAAAAGGYGPGQQGPYGPGGSAAAAAGPGSGGYGPGASAAAAAGGNGPGSGGYGPGQQGPGGSAAAAAGGYQQGPGGQGPYGPGASAAAAAGPGSGQQGPGAS

SEQ ID NO: 5 - protein, 603 aa, synthetic construct
  source 1..603: note = PRT1000
MHHHHHHSSGSSCGPGVFGPYGPGASAAAAAGINGPGSGVFGPGISGIYGPGVFGPGVFGPGSSAAAAAGPGIYGPGVFGPSASAAAAAGPGSGVFGPGASGIYGPGVFGPGVFGPGSSAAAAAGIYGSGPGVFGPYGSAAAAAGPGSGIYGIGPYGPGASGPGIYGPGVFGPSASAAAAAGSGVFGPGIYGPYASAAAAAGIYGSGPGVFGPYGPGISGSGVFGPGVFGPYASAAAAAGPGVFGPYGPGSSAAAAAGIYGYGPGVFGPYGPGASGINGPGSGIYGPGVFGPGISAAAAAGPGVFGPYGPGASAAAAAGIYGPGVFGPGIYGPGSSGPGVFGPYGPGSSAAAAAGIYGPGVFGPYGPGISAAAAAGIYVFGPGVFGPYGPGASGPGVFGPYGPGASAAAAAGPGIYGPGVFGPSASAAAAAGIYGSGPGIYGPYGPGISGPGSGVFGIGPYGPGASAAAAAGIYGPGVFGPYGPGISAAAAAGPGSGIYGPGASGINGPGSGIYGPGVFGPGISAAAAAGIYVFGPGVFGPYGPGASAAAAAGIYGSGPGVFGPYGPGISGSGVFGPGVFGPYASAAAAAGPGCSGVFGPGAS

SEQ ID NO: 6 - protein, 605 aa, synthetic construct
  source 1..605: note = PRT1001
MHHHHHHSSGSSCGPGVFGPYGPGASAAAAAGINGPGSGVFGPGISCGIYGPGVFGPGVFGPGSSAAAAAGPGIYGPGVFGPSASAAAAAGPGSGVFGPGASGIYGPGVFGPGVFGPGSSAAAAAGIYGSGPGVFGPYGSAAAAAGPGSGIYGIGPYGPGASGPGIYGPGVFGPSASAAAAAGSGVFGPGIYGPYASAAAAAGIYGSGPGVFGPYGPGISGSGVFGPGVFGPYASAAAAAGPGVFGPYGPGSSAAAAAGIYGYGPGVFGPYGPGASGINGPGSGIYGPGVFGPGISAAAAAGPGVFGPYGPGASAAAAAGIYGPGVFGPGIYGPGSSGPGVFGPYGPGSSAAAAAGIYGPGVFGPYGPGISAAAAAGIYVFGPGVFGPYGPGASGPGVFGPYGPGASAAAAAGPGIYGPGVFGPSASAAAAAGIYGSGPGIYGPYGPGISGPGSGVFGIGPYGPGASAAAAAGIYGPGVFGPYGPGISAAAAAGPGSGIYGPGASGINGPGSGIYGPGVFGPGISAAAAAGIYVFGPGVFGPYGPGASAAAAAGIYGSGPGVFGPYGPGISGCSGVFGPGVFGPYASAAAAAGPGCSGVFGPGAS

SEQ ID NO: 7 - protein, 1188 aa, synthetic construct
  source 1..1188: note = PRT587
MHHHHHHSSGSSGPGQQGPYGPGASAAAAAGQNGPGSGQQGPGQSGQYGPGQQGPGQQGPGSSAAAAAGPGQYGPGQQGPSASAAAAAGPGSGQQGPGASGQYGPGQQGPGQQGPGSSAAAAAGQYGSGPGQQGPYGSAAAAAGPGSGQYGQGPYGPGASGPGQYGPGQQGPSASAAAAAGSGQQGPGQYGPYASAAAAAGQYGSGPGQQGPYGPGQSGSGQQGPGQQGPYASAAAAAGPGQQGPYGPGSSAAAAAGQYGYGPGQQGPYGPGASGQNGPGSGQYGPGQQGPGQSAAAAAGPGQQGPYGPGASAAAAAGQYGPGQQGPGQYGPGSSGPGQQGPYGPGSSAAAAAGQYGPGQQGPYGPGQSAAAAAGQYQQGPGQQGPYGPGASGPGQQGPYGPGASAAAAAGPGQYGPGQQGPSASAAAAAGQYGSGPGQYGPYGPGQSGPGSGQQGQGPYGPGASAAAAAGQYGPGQQGPYGPGQSAAAAAGPGSGQYGPGASGQNGPGSGQYGPGQQGPGQSAAAAAGQYQQGPGQQGPYGPGASAAAAAGQYGSGPGQQGPYGPGQSGSGQQGPGQQGPYASAAAAAGPGSGQQGPGASGQQGPYGPGASAAAAAGQNGPGSGQQGPGQSGQYGPGQQGPGQQGPGSSAAAAAGPGQYGPGQQGPSASAAAAAGPGSGQQGPGASGQYGPGQQGPGQQGPGSSAAAAAGQYGSGPGQQGPYGSAAAAAGPGSGQYGQGPYGPGASGPGQYGPGQQGPSASAAAAAGSGQQGPGQYGPYASAAAAAGQYGSGPGQQGPYGPGQSGSGQQGPGQQGPYASAAAAAGPGQQGPYGPGSSAAAAAGQYGYGPGQQGPYGPGASGQNGPGSGQYGPGQQGPGQSAAAAAGPGQQGPYGPGASAAAAAGQYGPGQQGPGQYGPGSSGPGQQGPYGPGSSAAAAAGQYGPGQQGPYGPGQSAAAAAGQYQQGPGQQGPYGPGASGPGQQGPYGPGASAAAAAGPGQYGPGQQGPSASAAAAAGQYGSGPGQYGPYGPGQSGPGSGQQGQGPYGPGASAAAAAGQYGPGQQGPYGPGQSAAAAAGPGSGQYGPGASGQNGPGSGQYGPGQQGPGQSAAAAAGQYQQGPGQQGPYGPGASAAAAAGQYGSGPGQQGPYGPGQSGSGQQGPGQQGPYASAAAAAGPGSGQQGPGAS

SEQ ID NO: 8 - protein, 110 aa, synthetic construct
  source 1..110: note = PRT2882
MHHHHHHSSGSSCGPGVFGPYGPGASAAAAAGINGPGSGVFGPGISGIYGPGVFGPGVFGPGSSAAAAAGPGIYGPGVFGPSASAAAAAGPGCSGVFGPGASGFILGFIL

SEQ ID NO: 9 - protein, 202 aa, synthetic construct
  source 1..202: note = PRT2841
MHHHHHHSSGSSCGPGVFGPYGPGASAAAAAGINGPGSGVFGPGISGIYGPGVFGPGVFGPGSSAAAAAGPGIYGPGVFGPSASAAAAAGPGSGVFGPGASGIYGPGVFGPGVFGPGSSAAAAAGIYGSGPGVFGPYGSAAAAAGPGSGIYGIGPYGPGASGPGIYGPGVFGPSASAAAAAGPGCSGVFGPGASGFILGFIL

SEQ ID NO: 10 - protein, 313 aa, synthetic construct
  source 1..313: note = PRT2662
MHHHHHHSSGSSCGPGVFGPYGPGASAAAAAGINGPGSGVFGPGISGIYGPGVFGPGVFGPGSSAAAAAGPGIYGPGVFGPSASAAAAAGPGSGVFGPGASGIYGPGVFGPGVFGPGSSAAAAAGIYGSGPGVFGPYGSAAAAAGPGSGIYGIGPYGPGASGPGIYGPGVFGPSASAAAAAGSGVFGPGIYGPYASAAAAAGIYGSGPGVFGPYGPGISGSGVFGPGVFGPYASAAAAAGPGVFGPYGPGSSAAAAAGIYGYGPGVFGPYGPGASGINGPGSGIYGPGVFGPGISAAAAAGPGCSGVFGPGAS

SEQ ID NO: 11 - protein, 3550 aa, synthetic construct
  source 1..3550: note = PRT1186
MHSSGSSCGPGQQGPYGPGASAAAAAGQNGPGSGQQGPGQSGQYGPGQQGPGQQGPGSSAAAAAGPGQYGPGQQGPSASAAAAAGPGSGQQGPGASGQYGPGQQGPGQQGPGSSAAAAAGQYGSGPGQQGPYGSAAAAAGPGSGQYGQGPYGPGASGPGQYGPGQQGPSASAAAAAGSGQQGPGQYGPYASAAAAAGQYGSGPGQQGPYGPGQSGSGQQGPGQQGPYASAAAAAGPGQQGPYGPGSSAAAAAGQYGYGPGQQGPYGPGASGQNGPGSGQYGPGQQGPGQSAAAAAGPGQQGPYGPGASAAAAAGQYGPGQQGPGQYGPGSSGPGQQGPYGPGSSAAAAAGQYGPGQQGPYGPGQSAAAAAGQYQQGPGQQGPYGPGASGPGQQGPYGPGASAAAAAGPGQYGPGQQGPSASAAAAAGQYGSGPGQYGPYGPGQSGPGSGQQGQGPYGPGASAAAAAGQYGPGQQGPYGPGQSAAAAAGPGSGQYGPGASGQNGPGSGQYGPGQQGPGQSAAAAAGQYQQGPGQQGPYGPGASAAAAAGQYGSGPGQQGPYGPGQSGSGQQGPGQQGPYASAAAAAGPGSGQQGPGASGSGQQGPYGPGASAAAAAGQNGPGSGQQGPGQSGQYGPGQQGPGQQGPGSSAAAAAGPGQYGPGQQGPSASAAAAAGPGSGQQGPGASGQYGPGQQGPGQQGPGSSAAAAAGQYGSGPGQQGPYGSAAAAAGPGSGQYGQGPYGPGASGPGQYGPGQQGPSASAAAAAGSGQQGPGQYGPYASAAAAAGQYGSGPGQQGPYGPGQSGSGQQGPGQQGPYASAAAAAGPGQQGPYGPGSSAAAAAGQYGYGPGQQGPYGPGASGQNGPGSGQYGPGQQGPGQSAAAAAGPGQQGPYGPGASAAAAAGQYGPGQQGPGQYGPGSSGPGQQGPYGPGSSAAAAAGQYGPGQQGPYGPGQSAAAAAGQYQQGPGQQGPYGPGASGPGQQGPYGPGASAAAAAGPGQYGPGQQGPSASAAAAAGQYGSGPGQYGPYGPGQSGPGSGQQGQGPYGPGASAAAAAGQYGPGQQGPYGPGQSAAAAAGPGSGQYGPGASGQNGPGSGQYGPGQQGPGQSAAAAAGQYQQGPGQQGPYGPGASAAAAAGQYGSGPGQQGPYGPGQSGSGQQGPGQQGPYASAAAAAGPGSGQQGPGASELGQQGPYGPGASAAAAAGQNGPGSGQQGPGQSGQYGPGQQGPGQQGPGSSAAAAAGPGQYGPGQQGPSASAAAAAGPGSGQQGPGASGQYGPGQQGPGQQGPGSSAAAAAGQYGSGPGQQGPYGSAAAAAGPGSGQYGQGPYGPGASGPGQYGPGQQGPSASAAAAAGSGQQGPGQYGPYASAAAAAGQYGSGPGQQGPYGPGQSGSGQQGPGQQGPYASAAAAAGPGQQGPYGPGSSAAAAAGQYGYGPGQQGPYGPGASGQNGPGSGQYGPGQQGPGQSAAAAAGPGQQGPYGPGASAAAAAGQYGPGQQGPGQYGPGSSGPGQQGPYGPGSSAAAAAGQYGPGQQGPYGPGQSAAAAAGQYQQGPGQQGPYGPGASGPGQQGPYGPGASAAAAAGPGQYGPGQQGPSASAAAAAGQYGSGPGQYGPYGPGQSGPGSGQQGQGPYGPGASAAAAAGQYGPGQQGPYGPGQSAAAAAGPGSGQYGPGASGQNGPGSGQYGPGQQGPGQSAAAAAGQYQQGPGQQGPYGPGASAAAAAGQYGSGPGQQGPYGPGQSGSGQQGPGQQGPYASAAAAAGPGSGQQGPGASVDGQQGPYGPGASAAAAAGQNGPGSGQQGPGQSGQYGPGQQGPGQQGPGSSAAAAAGPGQYGPGQQGPSASAAAAAGPGSGQQGPGASGQYGPGQQGPGQQGPGSSAAAAAGQYGSGPGQQGPYGSAAAAAGPGSGQYGQGPYGPGASGPGQYGPGQQGPSASAAAAAGSGQQGPGQYGPYASAAAAAGQYGSGPGQQGPYGPGQSGSGQQGPGQQGPYASAAAAAGPGQQGPYGPGSSAAAAAGQYGYGPGQQGPYGPGASGQNGPGSGQYGPGQQGPGQSAAAAAGPGQQGPYGPGASAAAAAGQYGPGQQGPGQYGPGSSGPGQQGPYGPGSSAAAAAGQYGPGQQGPYGPGQSAAAAAGQYQQGPGQQGPYGPGASGPGQQGPYGPGASAAAAAGPGQYGPGQQGPSASAAAAAGQYGSGPGQYGPYGPGQSGPGSGQQGQGPYGPGASAAAAAGQYGPGQQGPYGPGQSAAAAAGPGSGQYGPGASGQNGPGSGQYGPGQQGPGQSAAAAAGQYQQGPGQQGPYGPGASAAAAAGQYGSGPGQQGPYGPGQSGSGQQGPGQQGPYASAAAAAGPGSGQQGPGASKLGQQGPYGPGASAAAAAGQNGPGSGQQGPGQSGQYGPGQQGPGQQGPGSSAAAAAGPGQYGPGQQGPSASAAAAAGPGSGQQGPGASGQYGPGQQGPGQQGPGSSAAAAAGQYGSGPGQQGPYGSAAAAAGPGSGQYGQGPYGPGASGPGQYGPGQQGPSASAAAAAGSGQQGPGQYGPYASAAAAAGQYGSGPGQQGPYGPGQSGSGQQGPGQQGPYASAAAAAGPGQQGPYGPGSSAAAAAGQYGYGPGQQGPYGPGASGQNGPGSGQYGPGQQGPGQSAAAAAGPGQQGPYGPGASAAAAAGQYGPGQQGPGQYGPGSSGPGQQGPYGPGSSAAAAAGQYGPGQQGPYGPGQSAAAAAGQYQQGPGQQGPYGPGASGPGQQGPYGPGASAAAAAGPGQYGPGQQGPSASAAAAAGQYGSGPGQYGPYGPGQSGPGSGQQGQGPYGPGASAAAAAGQYGPGQQGPYGPGQSAAAAAGPGSGQYGPGASGQNGPGSGQYGPGQQGPGQSAAAAAGQYQQGPGQQGPYGPGASAAAAAGQYGSGPGQQGPYGPGQSGSGQQGPGQQGPYASAAAAAGPGSGQQGPGASGQQGPYGPGASAAAAAGQNGPGSGQQGPGQSGQYGPGQQGPGQQGPGSSAAAAAGPGQYGPGQQGPSASAAAAAGPGSGQQGPGASGQYGPGQQGPGQQGPGSSAAAAAGQYGSGPGQQGPYGSAAAAAGPGSGQYGQGPYGPGASGPGQYGPGQQGPSASAAAAAGSGQQGPGQYGPYASAAAAAGQYGSGPGQQGPYGPGQSGSGQQGPGQQGPYASAAAAAGPGQQGPYGPGSSAAAAAGQYGYGPGQQGPYGPGASGQNGPGSGQYGPGQQGPGQSAAAAAGPGQQGPYGPGASAAAAAGQYGPGQQGPGQYGPGSSGPGQQGPYGPGSSAAAAAGQYGPGQQGPYGPGQSAAAAAGQYQQGPGQQGPYGPGASGPGQQGPYGPGASAAAAAGPGQYGPGQQGPSASAAAAAGQYGSGPGQYGPYGPGQSGPGSGQQGQGPYGPGASAAAAAGQYGPGQQGPYGPGQSAAAAAGPGSGQYGPGASGQNGPGSGQYGPGQQGPGQSAAAAAGQYQQGPGQQGPYGPGASAAAAAGQYGSGPGQQGPYGPGQSGSGQQGPGQQGPYASAAAAAGPGSGQQGPGASSGSSHHHHHH

SEQ ID NO: 12 - protein, 24 aa, synthetic construct
  source 1..24: note = His tag and start codon
MHHHHHHHHHHSSGSSLEVLFQGP